European Patent Application EP 4 289 858 A1, published December 13, 2023. Title: Novel antimicrobial peptide with excellent cytoplasmic elution effect of pathogenic microorganisms. Applicant: Cellicon Lab Inc. The sequence listing filed with the application follows.

SEQUENCE LISTING (16 sequences)

SEQ ID NO: 1 - protein, 12 aa, Artificial Sequence
  antimicrobial peptide 1
KKLFKKILKYLK

SEQ ID NO: 2 - protein, 12 aa, Artificial Sequence
  antimicrobial peptide 2
RRLFRRILRYLR

SEQ ID NO: 3 - protein, 12 aa, Artificial Sequence
  antimicrobial peptide 3
RFLFRLILRYLR

SEQ ID NO: 4 - protein, 12 aa, Artificial Sequence
  antimicrobial peptide 4
RRLFRLILRYLF

SEQ ID NO: 5 - protein, 12 aa, Artificial Sequence
  antimicrobial peptide 5
RKLFKRILRYLK

SEQ ID NO: 6 - protein, 12 aa, Artificial Sequence
  antimicrobial peptide 6
KRLFRKILKYLR

SEQ ID NO: 7 - protein, 12 aa, Artificial Sequence
  antimicrobial peptide 7
KRLFKRILRYLK

SEQ ID NO: 8 - protein, 12 aa, Artificial Sequence
  antimicrobial peptide 8
RKLFRKILKYLR

SEQ ID NO: 9 - DNA, 36 bp, Artificial Sequence
  polynucleotide encoding antimicrobial peptide
aaaaaactgtttaaaaaaattctgaaatatctgaaa

SEQ ID NO: 10 - DNA, 36 bp, Artificial Sequence
  polynucleotide encoding antimicrobial peptide
cgccgcctgtttcgccgcattctgcgctatctgcgc

SEQ ID NO: 11 - DNA, 36 bp, Artificial Sequence
  polynucleotide encoding antimicrobial peptide
cgctttctgtttcgcctgattctgcgctatctgcgc

SEQ ID NO: 12 - DNA, 36 bp, Artificial Sequence
  polynucleotide encoding antimicrobial peptide
cgccgcctgtttcgcctgattctgcgctatctgttt

SEQ ID NO: 13 - DNA, 36 bp, Artificial Sequence
  polynucleotide encoding antimicrobial peptide
cgcaaactgtttaaacgcattctgcgctatctgaaa

SEQ ID NO: 14 - DNA, 36 bp, Artificial Sequence
  polynucleotide encoding antimicrobial peptide
aaacgcctgtttcgcaaaattctgaaatatctgcgc

SEQ ID NO: 15 - DNA, 36 bp, Artificial Sequence
  polynucleotide encoding antimicrobial peptide
aaacgcctgtttaaacgcattctgcgctatctgaaa

SEQ ID NO: 16 - DNA, 36 bp, Artificial Sequence
  polynucleotide encoding antimicrobial peptide
cgcaaactgtttcgcaaaattctgaaatatctgcgc